European Patent Specification EP 4 382 600 B1, published March 4, 2026. Title: A double layer microsphere with oligonucleotide sequence for single cell sequencing. Applicant: MobiDrop (Zhejiang) Co., Ltd. The sequence listing filed with the application follows.

SEQUENCE LISTING (1 sequence)

SEQ ID NO: 1 - DNA, 35 bp, Artificial Sequence
  D1
  misc_feature (34)..(34): n represents any DNA sequence having a length of 4 -14 bp, and preferably any DNA sequence having a length of 6 -12 bp.
acactctttccctacacgacgctcttccgatctna